European Patent Application EP 4 527 830 A1, published March 26, 2025. Title: A method for producing various monomers for manufacture of synthetic resins from fatty alcohols. Applicant: Jungoh, Ahn. The sequence listing filed with the application follows.

SEQUENCE LISTING (2 sequences)

SEQ ID NO: 1 - DNA, 4496 bp, synthetic construct
  source 1..4496: mol_type = other DNA
attctgaaatgagctgttgacaattaatcatcggctcgtataatgtgtggaattgtgagcggataacaattcccctctagaaataattttgtttaactttaagaaggagatatacatatgacggaaaccatctcgaccgccgcagtgccgaccaccgacctggaagaacaagtcaagcgtcgcatcgaacaagttgtgagcaatgacccgcagctggccgcactgctgccagaggacagcgtcaccgaagctgttaacgaaccggatctgccactggttgaagtcatccgtcgtctgctggaaggctatggtgaccgtccggcattgggccagcgtgcattcgagtttgtcaccggcgacgacggcgcaacggttatcgcgctgaagcctgagtatacgacggtttcgtaccgtgagctgtgggagcgcgcagaggcaatcgcggcagcttggcacgagcaaggtattcgcgacggcgatttcgtggcgcaactgggttttaccagcaccgacttcgcgagcttagatgttgcgggtctgcgtctgggtaccgtgtcggtcccgttgcagaccggtgcgagcctgcagcagcgtaatgctattctggaagagactcgtccggctgtttttgcggcgagcattgaatacttggatgcggccgtggatagcgtgctggcgaccccgagcgtgagactgctgagcgtgtttgactatcacgcagaagtggactcacagcgcgaggcactcgaagccgttcgtgcgcgtctggagtccgcgggtcgtacgatcgtggtcgaggcccttgccgaagcgctggcccgtggtcgcgatctgccggctgccccgctgccgagcgcggaccctgacgcactgcgcctcctgatctacaccagcggtagcaccggtaccccgaagggcgcgatgtacccgcagtggttagtcgcgaacctgtggcagaagaaatggctgaccgacgacgtcatcccgagcatcggtgtgaattttatgccgatgagccatctggcgggcagactgacgctgatgggtaccttgagcggtggcggcacggcctactacattgccagcagcgacctgtctaccttctttgaagatattgcgctgatccgtccgtctgaagtactgtttgtcccgcgtgtggttgaaatggtgtttcagcgcttccaagcggaactggaccgttccctggccccaggcgagagcaacagcgaaattgctgaacgcattaaagtccgtattcgtgagcaagactttggtggccgcgtgctgtccgctggttccggcagcgccccgctgagcccggaaatgaccgaatttatggaaagcctgctgcaagttccacttcgtgatggttacggttcgaccgaggccggcggcgtttggcgtgacggtgttttgcagcgcccgccggtcacggattataaactggtagacgttcctgagctgggttacttcacgacggatagcccgcacccgcgtggtgagctgcgtctgaagtcagagactatgtttccgggttattacaagcgtccggaaacgaccgccgatgtgttcgatgatgagggctactataagaccggtgatgttgtggcggaactgggtccggatcacctgaagtatctggaccgcgttaaaaatgtgttgaaactggcacagggtgagttcgttgcggttagcaaactggaagctgcgtacacgggtagcccgctggttcgccaaattttcgtgtacggtaatagcgagcgtagctttctgctggcagtggttgtgccgactcctgaagtgttggagcgttacgccgactctccggatgcgctgaaaccgctgattcaggatagcctgcaacaagtggcaaaagacgcggaactgcagagctatgaaatcccgcgtgactttattgttgagactgtcccgtttactgtggagtcgggtttgctgagcgatgctcgtaagctgctgcgcccgaagctgaaagatcactacggcgagcgtctggaagccttatatgcagagctcgcggaaagccaaaacgaacgtttgcgccaactggcacgtgaggcagcgacgcgtccggttctggaaaccgttaccgacgcagcggctgcactgctgggtgctagcagcagcgacttggcgccagacgtgcgcttcattgatctgggtggcgattccctgagcgcactgagctacagcgagctgctgcgtgatattttcgaagttgatgtcccggtgggtgtgatcaacagcgtcgcgaatgatctggcagcaattgcgcgccatatcgaagcgcagcgtacgggtgcagcaacgcaaccgacgttcgcgagcgtccatggtaaagacgcgacggtgattacggcaggcgagctgaccctggataagtttctggacgagagcctgctgaaagccgcaaaagacgtacagccggcgactgccgacgttaagaccgtcctggtgaccggtggcaatggctggctgggtcgttggttggtgctggattggctggagcgcctggcgccgaacggtggcaaggtctatgcactgatccgcggtgcggacgcagaggccgcccgtgcgcgcttggacgctgtctacgagtccggtgatccgaagctgagcgctcactaccgtcaactggcccagcagtccttagaagtcatcgcgggtgacttcggcgatcaagacttgggtctgagccaagaggtgtggcagaaactggcgaaagacgtcgatctgattgttcattccggtgcgctggtcaatcatgtgttgccgtattcccagctgtttggcccgaatgttgctggcaccgcagagatcatcaaattggcaatttctgagcgcctgaagcctgtgacctatctgagcaccgtcggtattgctgatcagattcctgttaccgagttcgaagaggatagcgacgttcgtgttatgtccgcggagcgccagatcaacgatggttacgccaacggttatggtaacagcaaatgggcaggcgaagttctgctgcgtgaggcgcatgacctggccggtctgccggtccgtgtttttcgtagcgatatgatccttgcgcacagcgactaccatggtcaactgaatgttaccgacgtgttcacccgtagcatccagagcctgttgctgaccggcgtggcgccggcgagcttctacgaactggacgcagacggcaaccgccagcgcgcgcactacgatggtgttccgggtgatttcaccgcagcgtctatcaccgcaattggcggcgttaatgtcgtggatggttaccgttctttcgacgttttcaacccgcaccatgacggcgtcagcatggacacgtttgtcgattggctgattgacgccggttataagatcgcgcgcattgatgattatgaccagtggctggcgcgcttcgagttggctctgaagggtctgccggaacaacagcgtcagcaatctgtgctgccgctgttgaaaatgtatgagaagccgcaaccggcgatcgatggtagcgcgctgccgacggccgagttcagccgtgcggtccacgaagcaaaagttggcgactccggtgagattccgcacgtcacgaaagaactgattttgaaatacgcgtctgatatccagctgttgggtctggtctaataagaattcgaaggaggtaaaaaatgaaaatctacggtatctatatggatcgcccgctgtcacaagaagagaacgaacgctttatgtcctttatttcgccggagaagcgtgagaagtgccgccgtttctaccacaaggaagatgcgcaccgcaccctgctgggtgacgttctggtccgtagcgtcattagccgtcagtatcagctggacaaaagcgatatccgtttcagcactcaagagtatggcaagccgtgcatcccggacttgccggacgcgcatttcaatatctcccattctggccgttgggtcatttgtgcgtttgacagccagccgatcggtattgatattgagaaaaccaaaccgatcagcctggaaatcgctaagcgtttcttcagcaagaccgagtacagcgatctgctcgcaaaagacaaagatgagcagacggactatttctaccacctgtggagcatgaaagaatcctttatcaaacaagaaggcaagggtttgagcctgccgctggatagcttctctgtgcgtctgcaccaagacggccaggtgagcattgagctgcctgacagccatagcccgtgttacattaagacctacgaagttgacccaggttacaaaatggccgtgtgcgcagcgcacccggattttccggaagatattacgatggttagctatgaagaactgctgtaataagtcgacggatcggttgtcgagtaaggatctccaggctcgagcatcaaataaaacgaaaggctcagtcgaaagactgggcctttcgttttatctgttgtttgtcggtgaacgctctctgcccgggtgactgactgaaagctt

SEQ ID NO: 2 - DNA, 3787 bp, synthetic construct
  source 1..3787: mol_type = other DNA
attctgaaatgagctgttgacaattaatcatcggctcgtataatgtgtggaattgtgagcggataacaattcccctctagaaataattttgtttaactttaagaaggagatatacatatgaaagcggcagtcgtcaacgagttcaaaaaagcgttggaaatcaaagaagtggagcgccctaagttagaagagggcgaagtgctcgttaagatcgaggcctgcggcgtttgccataccgatcttcacgcagcccatggtgattggccgatcaaaccaaaattgccgttgattccgggtcacgaaggcgtcggtatcgtcgtcgaagtggcgaaaggtgtgaagtctatcaaggttggtgaccgcgtaggtattccgtggttgtactcggcgtgcggtgagtgtgagtattgcttgaccggccaggaaacgttgtgtccgcaccagttgaacggtggctatagcgtggatggcggctacgctgagtattgtaaggcgccagcagactacgtggccaagattccggataacttggacccggtggaagtcgccccgatcttgtgcgccggtgtgaccacctacaaggcattaaaagttagcggtgcaagacctggtgagtgggtggcgatttacggcattggtggtttgggtcacatcgcgttgcagtacgcaaaggctatgggtttgaatgtcgtggcggttgacattagcgatgagaaaagcaaactcgcaaaagatttgggtgccgacatcgcgatcaacggtttgaaagaggacccggttaaggcaattcacgaccaggttggcggcgtccatgctgcaatcagcgtcgccgttaacaaaaaggcattcgaacaggcgtatcagagcgtgaagcgtggtggtacgttggttgttgtcggtttaccgaatgctgatcttccgatccctattttcgatacggttttgaacggtgttagcgttaagggcagcatcgttggcacccgcaaagacatgcaagaagcgttggacttcgcggcgcgtggtaaggtccgcccgatcgtggaaacggcggagttggaagaaatcaatgaagtttttgagcgtatggagaaaggtaaaatcaatggtcgtattgtgttaaaattgaaagaagatcaccaccatcatcaccactaataacaaggaggtaaaaaatgcaaaaacaacgtactacctcccaatggagagaattggatgcagcccatcatttgcatccatttaccgacaccgcatccttgaatcaagctggcgcacgtgtgatgacccgtggcgagggcgtttacctgtgggattctgagggtaacaaaatcattgatggtatggccggtttgtggtgtgtgaacgtgggttatggtcgtaaagacttcgcagaagcagcccgtcgtcagatggaagaattgcctttctacaacactttcttcaaaactacccacccagctgtggtcgagttgtcttccttgttggccgaagttaccccagctggtttcgaccgcgttttctacaccaattcgggctccgagtctgttgacaccatgatccgtatggtgcgccgttattgggacgtccagggcaagcctgagaagaaaaccttgattggccgctggaatggttatcatggttccaccattggtggcgcatcgttgggcggtatgaaatacatgcacgaacagggcgatttgcctatcccaggtatggcccacattgagcagccttggtggtataagcacggtaaagatatgacccctgacgaatttggtgtggttgccgcacgctggttggaagaaaagatcttggagatcggtgccgataaggtcgcagcctttgttggcgagccaattcaaggtgcaggtggtgttatcgtcccacctgcaacctactggccagagatcgagcgtatttgccgtaagtatgacgttttgttggtcgccgatgaagtgatctgcggcttcggtcgcaccggtgagtggtttggtcaccaacactttggcttccagcctgacttgtttaccgccgcaaagggcttgtcttccggttacttgcctattggtgctgtttttgtgggtaaacgcgtcgcagaaggcttgattgccggtggcgactttaatcatggcttcacctactccggccatcctgtgtgcgcagcagtcgcacacgcaaatgtcgccgctttgcgcgacgaaggcattgtacagcgcgttaaagacgatattggtccatacatgcagaagcgctggcgtgaaaccttctctcgtttcgagcacgtcgatgatgtgcgtggcgttggtatggttcaagccttcactttggtcaaaaacaaggcaaagcgtgagttgtttcctgatttcggtgagatcggtaccttgtgccgtgacatctttttccgtaacaacttgattatgcgtgcatgtggtgatcacatcgtgtccgcaccacctttggttatgacccgtgccgaagtggacgagatgttggcagtggcagagcgctgtttggaagagtttgagcagaccttgaaagcccgtggtttggcctaataagaaggaggtaaaaaaatgatcatcggcgtccctaaagaaattaaaaacaatgagaaccgcgtcgcactcacgccgggtggtgtctcccagttgatctctaacggtcaccgcgtgcttgttgagactggtgccggcttgggtagcggctttgagaacgaagcgtacgagagcgcgggtgcagagatcattgcagatccgaaacaagtttgggatgcggagatggtcatgaaagttaaggaaccgttgccagaggaatatgtttacttccgtaagggcttggttctcttcacctatttgcacttggcggctgagccggaattggctcaggcgttgaaggacaaaggcgtgaccgccattgcgtacgaaaccgtaagcgagggtcgtaccttgcctttgcttacgccgatgtccgaggtcgcgggtcgtatggccgcacaaattggtgcgcagtttttggagaaaccgaagggtggcaagggtatcttgttggctggcgtgccgggtgtgagccgtggcaaggtgaccattattggtggcggtgttgtgggtaccaatgcagcaaagatggcagtcggcttgggcgcagacgtgacgattattgacttgaacgcggaccgtttgcgtcagctcgacgacatttttggtcatcagattaagaccctcatcagcaatccggtgaatattgcggacgccgtggcagaggccgatttgttaatctgtgcggtcttgattccaggcgctaaggcgccgaccttggtcaccgaagagatggtgaaacaaatgaagccgggtagcgtgatcgttgatgtcgcgatcgaccagggcggcattgtcgaaactgttgaccacattacgacccacgaccaaccgacctacgagaagcacggtgttgtccattatgcagttgcgaatatgccgggtgcggtcccgcgtacgtccaccatcgcattgaccaacgtgacggttccgtatgccttgcaaattgccaataagggtgctgtcaaagcattagcagataataccgccttgcgtgcgggtttgaacacggctaatggccacgtgacgtatgaagctgttgcgcgcgatttgggttacgaatacgtgccggcggagaaagcattgcaagatgagagcagcgtcgcgggtgcgcaccaccaccatcaccattaataatgactgactgactagcataaccccttggggcctctaaacgggtcttgaggggttttttg